European Patent Application EP 4 647 084 A1, published November 12, 2025. Title: 一种TSLP抗体治疗哮喘的方法. Applicant: 江苏恒瑞医药股份有限公司. The sequence listing filed with the application follows.

SEQUENCE LISTING (10 sequences)

SEQ ID NO: 1 - protein, 5 aa, Artificial Sequence
NYLIE

SEQ ID NO: 2 - protein, 17 aa, Artificial Sequence
VIDPGVGDTNYNENFKG

SEQ ID NO: 3 - protein, 10 aa, Artificial Sequence
EDNTGTAFDY

SEQ ID NO: 4 - protein, 11 aa, Artificial Sequence
KASQSVSSDVT

SEQ ID NO: 5 - protein, 7 aa, Artificial Sequence
YVSEHYT

SEQ ID NO: 6 - protein, 9 aa, Artificial Sequence
QQHHRFPLT

SEQ ID NO: 7 - protein, 119 aa, Artificial Sequence
EVQLVQSGAEVKKPGSSVKVSCKASGYTFSNYLIEWVRQAPGQGLEWIGVIDPGVGDTNYNENFKGRATLTADKSTSTAYIELSSLRSEDTAVYYCAREDNTGTAFDYWGQGTTVTVSS

SEQ ID NO: 8 - protein, 107 aa, Artificial Sequence
SIVMTQTPLSLSVTPGQPASISCKASQSVSSDVTWYLQKPGQSPQLLIYYVSEHYTGVPDRFSGSGYGTDFTLKISRVEAEDVGVYYCQQHHRFPLTFGQGTKLEIK

SEQ ID NO: 9 - protein, 449 aa, Artificial Sequence
EVQLVQSGAEVKKPGSSVKVSCKASGYTFSNYLIEWVRQAPGQGLEWIGVIDPGVGDTNYNENFKGRATLTADKSTSTAYIELSSLRSEDTAVYYCAREDNTGTAFDYWGQGTTVTVSSASTKGPSVFPLAPSSKSTSGGTAALGCLVKDYFPEPVTVSWNSGALTSGVHTFPAVLQSSGLYSLSSVVTVPSSSLGTQTYICNVNHKPSNTKVDKKVEPKSCDKTHTCPPCPAPELLGGPSVFLFPPKPKDTLYITREPEVTCVVVDVSHEDPEVKFNWYVDGVEVHNAKTKPREEQYNSTYRVVSVLTVLHQDWLNGKEYKCKVSNKALPAPIEKTISKAKGQPREPQVYTLPPSRDELTKNQVSLTCLVKGFYPSDIAVEWESNGQPENNYKTTPPVLDSDGSFFLYSKLTVDKSRWQQGNVFSCSVMHEALHNHYTQKSLSLSPGK

SEQ ID NO: 10 - protein, 214 aa, Artificial Sequence
SIVMTQTPLSLSVTPGQPASISCKASQSVSSDVTWYLQKPGQSPQLLIYYVSEHYTGVPDRFSGSGYGTDFTLKISRVEAEDVGVYYCQQHHRFPLTFGQGTKLEIKRTVAAPSVFIFPPSDEQLKSGTASVVCLLNNFYPREAKVQWKVDNALQSGNSQESVTEQDSKDSTYSLSSTLTLSKADYEKHKVYACEVTHQGLSSPVTKSFNRGEC